European Patent Application EP 4 768 506 A1, published July 1, 2026. Title: 靶向GPC3的分子探针以及用途. Applicant: 武汉睿迪辐生物科技有限公司. The sequence listing filed with the application follows.

SEQUENCE LISTING (12 sequences)

SEQ ID NO: 1 - protein, 8 aa, Artificial sequence
GFTFRSYA

SEQ ID NO: 2 - protein, 8 aa, Artificial sequence
ISGSGGRT

SEQ ID NO: 3 - protein, 19 aa, Artificial sequence
AKEYDFKTGWMHYYYGMDV

SEQ ID NO: 4 - protein, 5 aa, Artificial sequence
SSGYD

SEQ ID NO: 5 - skipped

SEQ ID NO: 6 - protein, 10 aa, Artificial sequence
QSYDSSLNAI

SEQ ID NO: 7 - protein, 126 aa, Artificial sequence
EVQLVESGGGLVQPGGSLRLSCAASGFTFRSYAMSWVRQAPGKGLEWVSAISGSGGRTYYADSVKGRFTISRDNSKNTLYLQMNSLRAEDTAVYYCAKEYDFKTGWMHYYYGMDVWGQGTTVTVSS

SEQ ID NO: 8 - protein, 106 aa, Artificial sequence
QSVLTQPPSVSGAPGQRVTISCTGSSSGYDVHWYQQLPGRAPKLLIYGSNNRPSGVPDRFSGSNSGTSASLAITGLQAEDEADYYCQSYDSSLNAIFGGGTKLTVL

SEQ ID NO: 9 - protein, 456 aa, Artificial sequence
EVQLVESGGGLVQPGGSLRLSCAASGFTFRSYAMSWVRQAPGKGLEWVSAISGSGGRTYYADSVKGRFTISRDNSKNTLYLQMNSLRAEDTAVYYCAKEYDFKTGWMHYYYGMDVWGQGTTVTVSSASTKGPSVFPLAPSSKSTSGGTAALGCLVKDYFPEPVTVSWNSGALTSGVHTFPAVLQSSGLYSLSSVVTVPSSSLGTQTYICNVNHKPSNTKVDKKVEPKSCDKTHTCPPCPAPELLGGPSVFLFPPKPKDTLMISRTPEVTCVVVDVSHEDPEVKFNWYVDGVEVHNAKTKPREEQYNSTYRVVSVLTVLHQDWLNGKEYKCKVSNKALPAPIEKTISKAKGQPREPQVYTLPPSRDELTKNQVSLTCLVKGFYPSDIAVEWESNGQPENNYKTTPPVLDSDGSFFLYSKLTVDKSRWQQGNVFSCSVMHEALHNHYTQKSLSLSPGK

SEQ ID NO: 10 - protein, 212 aa, Artificial sequence
QSVLTQPPSVSGAPGQRVTISCTGSSSGYDVHWYQQLPGRAPKLLIYGSNNRPSGVPDRFSGSNSGTSASLAITGLQAEDEADYYCQSYDSSLNAIFGGGTKLTVLGQPKAAPSVTLFPPSSEELQANKATLVCLISDFYPGAVTVAWKADSSPVKAGVETTTPSKQSNNKYAASSYLSLTPEQWKSHRSYSCQVTHEGSTVEKTVAPTECS

SEQ ID NO: 11 - protein, 234 aa, Artificial sequence
EVQLVESGGGLVQPGGSLRLSCAASGFTFRSYAMSWVRQAPGKGLEWVSAISGSGGRTYYADSVKGRFTISRDNSKNTLYLQMNSLRAEDTAVYYCAKEYDFKTGWMHYYYGMDVWGQGTTVTVSSASTKGPSVFPLAPSSKSTSGGTAALGCLVKDYFPEPVTVSWNSGALTSGVHTFPAVLQSSGLYSLSSVVTVPSSSLGTQTYICNVNHKPSNTKVDKKVEPKSCDKTHL

SEQ ID NO: 12 - protein, 254 aa, Artificial sequence
EVQLVESGGGLVQPGGSLRLSCAASGFTFRSYAMSWVRQAPGKGLEWVSAISGSGGRTYYADSVKGRFTISRDNSKNTLYLQMNSLRAEDTAVYYCAKEYDFKTGWMHYYYGMDVWGQGTTVTVSSGGGGSGGGGSGGGGSQSVLTQPPSVSGAPGQRVTISCTGSSSGYDVHWYQQLPGRAPKLLIYGSNNRPSGVPDRFSGSNSGTSASLAITGLQAEDEADYYCQSYDSSLNAIFGGGTKLTVLGHHHHHH